European Patent Application EP 4 410 814 A1, published August 7, 2024. Title: Peptide having hair loss preventing activity or hair growth promoting activity and use thereof. Applicant: CAREGENE CO., LTD. The sequence listing filed with the application follows.

SEQUENCE LISTING (15 sequences)

SEQ ID NO: 1 - protein, 8 aa, synthetic construct
KLQEHLDM

SEQ ID NO: 2 - DNA, 20 bp, synthetic construct
  source 1..20: mol_type = other DNA
ccagctattgtaacacctca

SEQ ID NO: 3 - DNA, 20 bp, synthetic construct
  source 1..20: mol_type = other DNA
ttcagatgtaggcagctgtc

SEQ ID NO: 4 - DNA, 25 bp, synthetic construct
  source 1..25: mol_type = other DNA
accagcagcgactctgaggaggaac

SEQ ID NO: 5 - DNA, 26 bp, synthetic construct
  source 1..26: mol_type = other DNA
tgaccctcttggcagcaggatagtcc

SEQ ID NO: 6 - DNA, 28 bp, synthetic construct
  source 1..28: mol_type = other DNA
accttcgttgccctctgtgccacagatg

SEQ ID NO: 7 - DNA, 21 bp, synthetic construct
  source 1..21: mol_type = other DNA
aggcccggaggcagtccgggt

SEQ ID NO: 8 - DNA, 20 bp, synthetic construct
  source 1..20: mol_type = other DNA
ggagccaaaagggtcatcat

SEQ ID NO: 9 - DNA, 20 bp, synthetic construct
  source 1..20: mol_type = other DNA
gtgatggcatggactgtggt

SEQ ID NO: 10 - DNA, 20 bp, synthetic construct
  source 1..20: mol_type = other DNA
ccaaatccgcaccaaggtca

SEQ ID NO: 11 - DNA, 21 bp, synthetic construct
  source 1..21: mol_type = other DNA
gtattgattgccaggaggggg

SEQ ID NO: 12 - DNA, 20 bp, synthetic construct
  source 1..20: mol_type = other DNA
cgcggcgtatccgtgtcctc

SEQ ID NO: 13 - DNA, 24 bp, synthetic construct
  source 1..24: mol_type = other DNA
agcctgttccgtctcaaacttggt

SEQ ID NO: 14 - DNA, 20 bp, synthetic construct
  source 1..20: mol_type = other DNA
cggtcaagtcggaaaattca

SEQ ID NO: 15 - DNA, 20 bp, synthetic construct
  source 1..20: mol_type = other DNA
gaggagctgggatgtggtaa